European Patent Application EP 4 276 110 A1, published November 15, 2023. Title: An anti-PD-L1/anti-4-1BB bispecific antibody in the form of an anti-PD-L1/anti-4-1BB natural antibody structure-like heterodimer and its preparation thereof. Applicant: BEIJING HANMI PHARMACEUTICAL CO., LTD. The sequence listing filed with the application follows.

SEQUENCE LISTING (26 sequences)

SEQ ID NO: 1 - DNA, 321 bp, Artificial Sequence
  light chain variable region
gacatccagatgacccagtccccttcctccctgtccgcctctgtgggcgacagggtgaccatcacctgcaaggcctcccaggatgtgcacaccgccgtggcttggattcagcagaagcccggcaagtcccccaagctgctgatctactccgcctccaaccggtacaccggcgtgcctagcaggttcagcggaagcggcagcggcaccgacttcaccttcaccatctcctccctgcagcctgaggacatcgccacctattactgccagcagcactacatcacccccctgaccttcggccagggcaccaagctggagatcaag

SEQ ID NO: 2 - protein, 107 aa, Artificial Sequence
  light chain variable region
DIQMTQSPSSLSASVGDRVTITCKASQDVHTAVAWIQQKPGKSPKLLIYSASNRYTGVPSRFSGSGSGTDFTFTISSLQPEDIATYYCQQHYITPLTFGQGTKLEIK

SEQ ID NO: 3 - DNA, 321 bp, Artificial Sequence
  light chain constant region
cgtacggtggccgcccccagcgtcttcatttttccaccctctgacgaacagctgaagtcagggacagcttccgtggtctgtctgctgaacaatttttaccccagggaggccaaagtgcagtggaaggtcgataacgctctgcagagcggaaattctcaggagagtgtgacagaacaggactcaaaagattccacttatagcctgtctagtaccctgacactgtccaaggcagactacgaaaagcataaagtgtatgcctgtgaggtcacacatcagggtctgtcaagccccgtcactaagtccttcaaccggggagaatgc

SEQ ID NO: 4 - protein, 107 aa, Artificial Sequence [sequence omitted]

SEQ ID NO: 5 - DNA, 351 bp, Artificial Sequence
  heavy chain variable region
gaagtgcagctggtgcagtccggcgccgaggtgaagaagcctggctcctccgtgaaggtgtcctgcaaggcctccggcttcaacatcgaggacacctacatccactgggtgaggcaggctcccggacagggactggagtggatgggcaggatcgatcccgccaacgccaacaccaagtacgaccccaagttccagggcagggtgaccatcaccgccgataccagcaccaacaccgcctacatggagctgtcctccctgaggtccgaggacacagccgtgtactactgtggcaggggactgggcgcctggtttgcctactggggacagggcaccctggtgaccgtgtcctcc

SEQ ID NO: 6 - protein, 117 aa, Artificial Sequence
  heavy chain variable region
EVQLVQSGAEVKKPGSSVKVSCKASGFNIEDTYIHWVRQAPGQGLEWMGRIDPANANTKYDPKFQGRVTITADTSTNTAYMELSSLRSEDTAVYYCGRGLGAWFAYWGQGTLVTVSS

SEQ ID NO: 7 - DNA, 990 bp, Artificial Sequence
  heavy chain constant region
gctagcacaaaaggaccttccgtgtttccactggcaccctctagtaagagtacttcaggaggaaccgcagcactgggatgtctggtgaaggactacttcccagagcccgtcaccgtgtcttggaacagtggagcactgacctccggggtccatacatttcctgccgtgctgcagtcatccggtctgtatagcctgagctctgtggtcacagtcccaagttcatccctgggcacccagacatacatctgcaacgtgaatcacaaaccttccaatactaaggtcgacaagaaagtggaacccaagtcctgcgataagacccacacatgccctccctgtcctgctcccgaactgctgggaggaccctccgtcttcctgttcccccccaagcccaaagacacactgatgatcagcaggacccctgaagtgacctgcgtggtcgtggacgtgagccacgaggaccccgaggtcaagtttaactggtacgtggacggcgtggaggtccacaacgccaagaccaagcccagggaggagcagtacaacagcacctacagggtcgtgtccgtgctgaccgtgctccaccaagattggctcaacggcaaggagtataagtgcaaagtcagcaacaaggccctccccgcccccatcgagaaaaccatcagcaaggccaagggccaaccgcgggaacctcaagtgtataccctccctcccagccgggatgagctgaccaagaaccaagtctccctcttgtgcctggtcaagggattctacccttccgacattgccgtcgaatgggagagcaatggccagcccgagaacaactacaagacaaccccccccgtcctgcgcagcgacggatccttcttcctgtactccaagctcaccgtggacaagagccggtggcaacagggcaacgtgttctcctgtagcgtgatgcacgaagccctccacaaccactatacccagaagagcctgagcctcagccccggcaaa

SEQ ID NO: 8 - protein, 330 aa, Artificial Sequence
  heavy chain constant region
ASTKGPSVFPLAPSSKSTSGGTAALGCLVKDYFPEPVTVSWNSGALTSGVHTFPAVLQSSGLYSLSSVVTVPSSSLGTQTYICNVNHKPSNTKVDKKVEPKSCDKTHTCPPCPAPELLGGPSVFLFPPKPKDTLMISRTPEVTCVVVDVSHEDPEVKFNWYVDGVEVHNAKTKPREEQYNSTYRVVSVLTVLHQDWLNGKEYKCKVSNKALPAPIEKTISKAKGQPREPQVYTLPPSRDELTKNQVSLLCLVKGFYPSDIAVEWESNGQPENNYKTTPPVLRSDGSFFLYSKLTVDKSRWQQGNVFSCSVMHEALHNHYTQKSLSLSPGK

SEQ ID NO: 9 - DNA, 321 bp, Artificial Sequence
  light chain variable region
gacatccagatgacccagagccctagcagcctgagcgccagcgtgggcgacagagtgaccatcacctgcagagccagccaggacatcagcaattacctgaattggtaccagcagaagcctggcaaggtgcctaagctgctgatctaccacaccagcagactgcacagcggcgtgcctagcagattcagcggcagcggcagcggcaccgacttcaccctgaccatcagcagcctgcagcctgaggacgtggccacctactactgccagcagggccacaccctgcctagaaccttcggcggcggcaccaaggtggagatcaag

SEQ ID NO: 10 - protein, 107 aa, Artificial Sequence
  light chain variable region
DIQMTQSPSSLSASVGDRVTITCRASQDISNYLNWYQQKPGKVPKLLIYHTSRLHSGVPSRFSGSGSGTDFTLTISSLQPEDVATYYCQQGHTLPRTFGGGTKVEIK

SEQ ID NO: 11 - DNA, 357 bp, Artificial Sequence
  heavy chain variable region
caggtgcagctggtgcagagcggcgccgaggtgaagaagcctggcagcagcgtgaaggtgagctgcaaggccagcggctacaccttcaccagctactggatcaattgggtgagacaggctccgggccaagggctggagtggatgggcaatatctaccctagcgacagctacaccaattacaatcagaagttcaaggacagagtgaccatcaccgccgacaagagcaccagcaccgcctacatggagctgagcagcctgagaagcgaggacaccgccgtgtactactgcgccagactgtactacggcagcagccctttcgactactggggacaaggcaccaccgtgaccgtgagcagc

SEQ ID NO: 12 - protein, 119 aa, Artificial Sequence
  heavy chain variable region
QVQLVQSGAEVKKPGSSVKVSCKASGYTFTSYWINWVRQAPGQGLEWMGNIYPSDSYTNYNQKFKDRVTITADKSTSTAYMELSSLRSEDTAVYYCARLYYGSSPFDYWGQGTTVTVSS

SEQ ID NO: 13 - DNA, 990 bp, Artificial Sequence
  heavy chain constant region
gctagcacaaaaggaccttccgtgtttccactggcaccctctagtaagagtacttcaggaggaaccgcagcactgggatgtctggtgaaggactacttcccagagcccgtcaccgtgtcttggaacagtggagcactgacctccggggtccatacatttcctgccgtgctgcagtcatccggtctgtatagcctgagctctgtggtcacagtcccaagttcatccctgggcacccagacatacatctgcaacgtgaatcacaaaccttccaatactaaggtcgacaagaaagtggaacccaagtcctgcgataagacccacacatgccctccctgtcctgctcccgaactgctgggaggaccctccgtcttcctgttcccccccaagcccaaagacacactgatgatcagcaggacccctgaagtgacctgcgtggtcgtggacgtgagccacgaggaccccgaggtcaagtttaactggtacgtggacggcgtggaggtccacaacgccaagaccaagcccagggaggagcagtacgccagcacctacagggtggtcagcgtgctgaccgtgctgcaccaggattggctcaacggcaaggagtacaagtgcaaagtctccaacaaggccctgcccgcccccatcgagaagaccatctccaaggctaagggacagcccagggagccccaagtgtacaccgagcctcccagccgggatgagctgaccaagaaccaagtctccctcacctgcctggtcaagggattctacccttccgacattgccgtcgaatgggagagcaatggccagcccgagaacaactacaagacaaccccccccgtcctggatagcgacggatccttcttcctgctctccgtgctcaccgtcgacaagagcagatggcagcagggcaacgtgttcagctgtagcgtgatgcacgaggccctgcacaaccactacacccagaagagcctgtccctcagccccggcaag

SEQ ID NO: 14 - protein, 330 aa, Artificial Sequence
  heavy chain constant region
ASTKGPSVFPLAPSSKSTSGGTAALGCLVKDYFPEPVTVSWNSGALTSGVHTFPAVLQSSGLYSLSSVVTVPSSSLGTQTYICNVNHKPSNTKVDKKVEPKSCDKTHTCPPCPAPELLGGPSVFLFPPKPKDTLMISRTPEVTCVVVDVSHEDPEVKFNWYVDGVEVHNAKTKPREEQYASTYRVVSVLTVLHQDWLNGKEYKCKVSNKALPAPIEKTISKAKGQPREPQVYTEPPSRDELTKNQVSLTCLVKGFYPSDIAVEWESNGQPENNYKTTPPVLDSDGSFFLLSVLTVDKSRWQQGNVFSCSVMHEALHNHYTQKSLSLSPGK

SEQ ID NO: 15 - protein, 10 aa, Artificial Sequence
  PD-L1 HCDR1
GFNIEDTYIH

SEQ ID NO: 16 - protein, 17 aa, Artificial Sequence
  PD-L1 HCDR2
RIDPANANTKYDPKFQG

SEQ ID NO: 17 - protein, 8 aa, Artificial Sequence
  PD-L1 HCDR3
GLGAWFAY

SEQ ID NO: 18 - protein, 11 aa, Artificial Sequence
  PD-L1 LCDR1
KASQDVHTAVA

SEQ ID NO: 19 - protein, 7 aa, Artificial Sequence
  PD-L1 LCDR2
SASNRYT

SEQ ID NO: 20 - protein, 9 aa, Artificial Sequence
  PD-L1 LCDR3
QQHYITPLT

SEQ ID NO: 21 - protein, 10 aa, Artificial Sequence
  4-1BB HCDR1
GYTFTSYWIN

SEQ ID NO: 22 - protein, 17 aa, Artificial Sequence
  4-1BB HCDR2
NIYPSDSYTNYNQKFKD

SEQ ID NO: 23 - protein, 10 aa, Artificial Sequence
  4-1BB HCDR3
LYYGSSPFDY

SEQ ID NO: 24 - protein, 11 aa, Artificial Sequence
  4-1BB LCDR1
RASQDISNYLN

SEQ ID NO: 25 - protein, 7 aa, Artificial Sequence
  4-1BB LCDR2
HTSRLHS

SEQ ID NO: 26 - protein, 9 aa, Artificial Sequence
  4-1BB LCDR3
QQGHTLPRT